European Patent Application EP 4 484 575 A1, published January 1, 2025. Title: Markersequenzen zur Diagnose und Therapiesteuerung von Patienten mit Testosteron-Defizienz. Applicant: cerascreen GmbH. Application EP, filed June 30, 2023. The sequence listing filed with the application follows.

SEQUENCE LISTING (12 sequences)

SEQ ID NO: 1 - DNA, 3054 bp, Homo sapiens
  source 1..3054: mol_type = genomic DNA
cggatcatcacagcccctagggatttgttgaatgacctttggcaaatcacttcccttctctgggcctgtagttcttggctgaatatgagggaatggatttcaaattatgctccatgtaatacccgtgtttttacctctgtaaacagatttttttgttttttttgagacggagtctcgttctgtcccccgggctggagtgcagtggcgcgatctcggctcactgcaacctccgcctcccgggttgacgccattctcctgcctcagcctccctagtaggtgggactacaggcgcccgccaccacgccgcccggctaattttttttttctttttctttttctttttttttttttgtatttttagtacagacagggtctcactgtgttagccaggatggtctcgatctcctgaccttgtgatccgcccgcctcggcctcccaaattgctgggattataggcgtgagccaccgcgcccggccccaacagatttttaaagatggtcttttcccaatttgtggaaatgttttaacagaatgctctcaatatttttcgcccatgtgattcttagattcatgtgaatctaacacaacgtatctgatactgttcccaacaggaaccagggtggcagggctagatgtcctctcaccagactgcccagtgaaggtgctgtcactttgatgaattatcaaggctttgtagtgggtcttctactggacaaaggacaaactggagactccctggatcaaatgtgttggtgaggcactgaatctgattgctgaaaggtgattcagctgcaagttaggcatcagtttagggttttctaggcttggcatctaaagggagtgcctgctgtagctgaaacctcataggccttctcttccttccgaattgttttcaaggccttgggggtacagagacttagagaaaatacatagttgtgcctcagactgatgggcctcatctgtttaatggagaaacaccaagcacactcagtctgggcggaattttagagctccatagtataaccactatctagctacatgtggcaattgagcatttgaaatgtggctagactgaattgaaatgtgctgtataaaatatacacttaatttcaaagacaatatttttaaaatgtaaaatatttcagtaatttaaaaatatggtttaaatattttagatatgttgggttaaataaaatatattagtaaaatatttcacttgttttttgacctcttaaatgtggctgctagaaaatgttatagtgctgtcaggaagtgctgttctggaatacagaatgtggctgccgtgagtggagtgtgactatgagatagtcgcctgactggagacaatgaagcctcaggccaaggtaagagggctgacaaggaagaactggcacaactagagccgaatgtttgggggaggtatatgtctgccaaaaaatgaatataatttcaggtgactcaatagaagtggagggatcagtttctcttgttctgccctgctcttatctaggtaactcttacttttcctttaggtcagggttcttctaagccagaaaaccttcactgacttaagtgcactcctttctatgtttgcatagatctctttcttaactttaccccattatagtaaaattatgttttcacatttgcctttatacccaaacctccaccaaaatattgtgagctctctgagggtaaggactttgtcttattattgttatacctggagacagattaaaacaatatgatgtttgtggggaccagggaaaaggggaatgggagaggctcctctggttagtctaaaagaaaagtatcaggcacctacttgaatcctcatttgatttctttctgaccatgagaggggatgctgagatgcccaaagatgtgcaaatggcgggatccggcgcaccatagtaggcaggggagtgaagatttctcacctcgggtcttcctagaccttcaggtcacacgggaattgttctgtttatagacggcgctggccttagtactcactctccctctattttccttgcttccttataactaggtttccctactcacttcctcaaaaagagtgatgtaggtccacgtgtaccctcccaactggcctgggtcctctcccttctttgtaaggcctgaaaaattccctggtgggggatggttagaaaaggaagaggaaccttctttgtaagtgtgcaagtcagaaggggagggagaaaagtgacaatttatatatctgggacaaatatatcttggacccaggttttgccacctgtctgcatccccccatgccctttcccctccagtgatcaaatagctctctggatgccccttaattcttccaccccatccattctgatctacccagcacttgcctaggcaacaccagtccaggagaacaaatggagttatgcacaacattggtgatttccttgtattgtggctccagtggttatggctggggacacacacatccttccagttatttctgagcatactctggaaacgtcttatgagccctcttctttattgtgtgcacccactaggatgctccctcctactcagccctgtttagtgggatttttcagcccactgtaaagcctactgctgcctgtaaagccacctaagtgcatcacttgctggtgttcaccatgataacaacaatttatggggacagaatatgtttctagagctgctggtgccactgctgatgttactgggttccctgaaataaaacaccacagtgcaggtgagtaccaaagtggggagaatttttagttccttttagaggtgctaaatcaatattgttgatttcccagtaccttagaatatttaatgaaaacaggtcaggtgcagtggctcacgcctgtaatcccagcactttgggaggccaaggcaggtagatcacttgaggtcaggagttcaagaacagcctggccaacatggtgaaaccccatctctactaaaaatacaaaaattagcagggcgtggtggcaggcacctgtaatcccagctactccggaagctgaggcaccagaatcgcttgaactcagg

SEQ ID NO: 2 - DNA, 3146 bp, Homo sapiens
  source 1..3146: mol_type = genomic DNA
cggtgggtctgtgacgactgcgatcagcaccacgagctaaagctcagctcgagccggaacacagaccagaagagtgtgtagttgcaagacttaatagagtgaaaacagaactcccatacaaaggagggaccaaaagggggttgcccaatccagctcgaatgcctgggtttatatccccatcattgtccctccccctgtgctctcaggcgatagctgatttgactgtttctttacctcctgcttttagcctaattggtatttcagtgagctccctttactacctgattggtcaggtgtgagctgagttagaagcccggtgtttaaaggtgggagtggtcaccttccccagctagggttaggaattcttatttggcctaggaaatccagctagtcctgtctgtcataacctcctgggctcctgtttgcctctctccctccagctcctttgctcttggtggcctctgattggggccaacactacaagcaaggtcaagcgcaggtccgtgtctcccctctcccatcctaaggcttcccaggaccagggccctccttcattttcttccttgaccctgatgctgaggagagggctgggaggcagcctgagctgtggaaaggctgggttgagattctagctcggccatttcctagcatgtgactccggggatgggacacaccctctccgagcctgttccctggttttaagatggggctcagggcatttcacaggcgcacatgggacagcatgaatgcacgtagtaggcctcccccagcttaacgagtggaggcccatctgttgcactcttgtctctgggaatatccttgtgggccccacagagaagccccaggtgtcttttcagagcccaccgttccttgtgaacagcatcacaccgggtgctaggggcgcaaagatgtggtcttagtaaaaacgaaattcctttgccttggtctgactcattctttccctaagatgtggccatttacaaagctctcttggagtcttcattgcttagatagggcagttctcttttatttatagcctagggactggacccaaggggcctaataaatgtttaaaataaccacagcccagccacctgaagcactgccccttcagccgccccctaggccaggcctttagatttggttccctctgggtggggggcattatcggggaatcagatgcggccatcagacatccagcagctacttggggatgcctcaagacacctgggctcagcacagcttctggcactcagcacctctccctcctgctggtcctgttcctcttccaagggctctcagcccaaagaatgggtccaggaagaaacacagcagtgtgtctgcattcccccctcacctcaccctcctccgcccagtcccatccatcagcaagtcccgcctgctctacgtgggttcctacagccctcctcctctccattcccatcccaccccatccaaggcgccgccatcccctgcctggtctccctcttgcacagcagcccctccagtgggtcttccttgcagcagccagagggagcccgtgtgagtgcgagcctgaccccgtggctgtgctcatatcaagcctaaaggcctcggccaggcacggtggctcatgcctgtaatcccagcactttgggaggccgaggcaggcagatcacctgaggtcaggagttcaagaccagcctggccaacctggtgaaaccccacctctactaaaaatacaaaaattagccaggcatggtggcgcatgccagtagtcccagctacttgggaggctgagggaggagaatcgcttgaacccgggaggcggaggttgcagtgagccgagatcgcgccactgcactccagcctgagggacagagcaagactctgtcaaaaaaaaaaaaagtataaaggcctcgtgcagcctccttacactgcaaccacggtgaccttcattcagttccccaaagcagccatgccctccccaacctccaggcctttgcacatgctgccaggatgatgcctacgcatcccccagacctcaatcacacctcagagaggtcttcccagccccttctccccaaaggtcagtggccctgtagtccctgtcatggccccctgcagctttctgtcaagtactaatcagcgttgggggtggcagcatatttaggggctgagtgatgtctggttcttgtgtctataagcttgaagaaggtagagacagcatctgtctgattcattgctgcttctggctcctgacaggtagtaggtactcaaaaaagtatttgttgagcaaatttggattgctaacagatgccaacactgtgctgctgacagcaaggtgacatggctgtctgtggagccacctgcccctaaatatggccgatgcggtcgacagaataatgaccccctgccccctgtgatgtctaggtccctgtccctgatgtgtgtggccgtgttaccttgcattcaaaaggaactttgcaaatgtgattacattaaggatctcgagatggggagaggatcctgggttagccaggtggactggatgaaatcacaagagttcctgtaagagagaggtggaggccaggcacagtggctcacgcctgtaatcccagcactttgggaggctgaggcgggggcggggggggggggagagaggggagggggggaggggggagggggggggtggatcatgaggtcaggagttcgggaccagccttgccaatatggtgaaaccccatctctactaaaaatacaaaaattagctggagtggtggcacgcacctgtagtcacagctactcgggaggctgaggcagaataattgcttggacctgggagatggaggttggagtgagccgagatcgcgccactgcactccagcctgggtaacagagtgagactctgtctcaaaaaataaaaaaagagagaggtggaggtcagagaagggggaagctgctggctttggaactgggagaaggggccacaagcctaggcagcgcctagaagctgaaaaaggcaagaaaatgcattctcccaagaacacagcccgttttagacttctgacctccaaaagcataagacaataaatgtgtgttggtttaagccattcccgttgtgataatttgttacagcagccacaggaaattaatacagccgtcaa

SEQ ID NO: 3 - DNA, 3071 bp, Homo sapiens
  source 1..3071: mol_type = genomic DNA
cgagaaaagatattcaagagatggcgagggttcagagccagaggccactgagagatgagatagtgattctgaaagtgtagtcctgaactggtagtgtcagcatcactttggaacttataaaaacgcaaactcttagttcccaccccagacatactgaatcagaaagtctggtcatgggatccagaaatctgcatttcaacaggcattcaggtgattctgatgcacactgaagtgtgaggaccattggatacaggatgagaactccaggaggccattttgactcttgaaaaagtaattctagttggatgaggcaggggagacgagggtacaggcaaatagtgacatgaagacaagtctcactgagtgaggatggggtttgggagccaagagctgggggttgggtccctgggagcagaggttgaggtgaacagagtgcaacgttgtgggagaggtctggggcccttacctggatgaccatgggctgcagcttcccattgggctccatcttcagcataacgaggggggcagccaggtattgcttctctcctcggatcacgttggctggaattccatccagaaggatgaagtcagcttcaaacagggaaccattctggggacaggagggatgtatccatttttagagttcaaagtctacccccagggggccggggcaaagggcaagagatttagtctagcttcttgccattctcctgcatcagtaccggagccctgttgggagaactagagcccctggtccagttcctctcatcttaaagtgaagaaacagtctggtgagggtagatgtcttgtgtgtggatgtggtggcagatctgggtttggaaccaggcctgctcaatccagttggcatcacaggcattgtaaactgaccacctgtcaaatggccaggcccctttctgatcattcccgaatggtctgcgctctggttttggctcctatcagctcagcaaatgctctttcattccctattcaaatctcacatcctctgccaaatattccagagagcttcccctactacccctgccaccgcatacagcacacacatgcatacgcacacattttgcctaggcttgtcctcagtacagtccattgcttccaaaccccgctctctttttctagaaagcctccccgattctccccacctgatggcacttcctcacttttctccctgcccatgaacactggagtccagaacactgcggccaggcaatgtcactgttcctgctaacatctccagcccctctctgtgtgctggggatccattctattttccccttcctgctgggagctcctcatagtttcttcccctacatattttatttctgtatttttccagcacaggactgcaccaaggggcaatgcagtactgcagccttcctctgactcagtttggattctctctgtccgttctcaccacactactaaggagagaacagtgccaggcaggggaaggagaggtacctgaagttctttctccagttgagcctgaagctcttccatccccgagggcagcactagcctggagggcagagaggtcgagcgtctcaacagcatggggttggcaccattgaggaactggtagctgaacaactcatcatcctgccagcactggcgaaccttctctttggtgggcggtgaaaggaggatatatgtaccacagcctgcatatcccttctccaaaatctaccccaggggttcaggtatataaccctccctgaacccagcttctgcgttttcattctcaaggcctctctgagttgaccagatatgataaggtctcttcttgcaaagagttacgggggactgtggagtgtgatgagtcatccagaggggccattaagggattatggagacctcggggaaccactgaccagccagggcactcttctggccccagaagatctgatcaaagtcttctaggcagttccaggagctcaggagggtgtaaacacgtttgagggccatctccagagccctaggacaggtattgaggcttaactcatcagctgatccctcagtccctcaccgtctatcatcattcttggccctcccagcccttatttcactccgaggtctagcctttttctcaccctgccttcagtgtccattcaaagtccagcctcttctcctcatggaatctcatatttggaggtagatcatccttacggtctgcagcgatggtcaggggtaacccttccttccaggtggcccagctaggagttggggacaaagcttcaggaaggatgtcatggtcagtgatggggccaggggcaggggcaggggcagggaaggggtgggacagtggtggcggggttagtttaaggggtgggtggtcaccagtagatctgctgtctgtctttcagttccttctctcgatgcttctggaacatgtccaaagcattgtctcctggcaggcgggctggggagacatcaagacaattggcctcacggctctgtctggtcctatgcccgcctcttgtcctcatctccctgtggttagccgtattccatgttttcagccatgcactgttgcttttatctctggctttgcctcatttgattatccaccagacacgtttatcccatctttgccaactttgcactcctgctttctcttatttcagccctcatcctttgcctgtagataaaaacctcctgtttgccaccatttcttgctccttcactcatcttcccctacctggccttacttcatcaatatctatggttggaaaaaaatcaccttaattaaggtgatgaaatcttagtcacctatacacctacacctactgtctactacagattgctttgattaatttcacatcttaaacctcacctgccacgccttcacctgtcctcaaaagattctacatttgcttttttttttttaaacctcatctttctggatttactatcataatctgtatctatggacttattctgggtcttttctgcatttacactcacctgtctcaaagtcatagatttgatgttccatccctactgccctcactcatctctggattcatctctcttttactcattacccatggtta

SEQ ID NO: 4 - DNA, 1711 bp, Homo sapiens
  source 1..1711: mol_type = genomic DNA
cgctgtcacagagctgactgatagagcttattccagggcatccttaccattcatcattgtctcactggctcctttccaaaagcttcctccattaagagggtcagagcctcagcttcctttctttctagtgacaatttcctttgttttaggggattttaaattagggtgctgaaggcctggaagaacatgggtgggaagagaatgtaactctaagtcatgtgtgtcattttcctttggggtgagagagtggctgtttgtgtaatgagacctttctctgcataacttccttttgtaagacctcaagggcctccaccagcaggtaatatttcagccatgatccagtgtggggaggcacaggtataagagggaagagcatgagctgagtgtacctgaccacagtggtccatgttcatggcctatttgctgctatgaggatcaagacttaggggagaagtttgccagtttctaggaatctccagacattgttccccagaaccaagccttaactttggtggcatcttcttgtgaaatgtggagccagaaccacagcttaaatgttagacactaggatgatgcccactttgtgccacatgatggtggctactgcctgtaagcattttccagtgactgaaagaggctgctagtggtcgggaagagatatcatccaatttcctaaaaagactgaacccttcatattccccagaagaataacagctgttccccacctcccacacatctgcatcaagctgaagttctgtgtcctcatgagctgatttcacctttgcacagatcttgggggaggtgatgacaatacaccctggacctcaactttctctgtctgaagctgcagggggcccctgaagggtgggggagatggcaggcccaccaggataccctgtgctgatcaatgctcttctctcttctccagggcttctgcactgactcctgagactattttaactaggattggttatcactcttctgtgatgcctgcttatgcctgcccagaattcccagctgcctgtgtcagcttgtccccctgagatcaaagtcctacagtggctgtcacgcagccaccaggtcatctcctttcatccccaccccaaggcgctggctgtgactctgcttcctgcactgacccagagcctctgcctgtgcatggccagctgcgtctactcaggtcccaaggggtttctgtttctattctttcctcagactgctcaagagaagcacatgaaaaacattacctgactttagagcttttttacataattaaacatgatcctgagttatctgtattctgaactttcttaattgagaagaggcaggaaatcactgcagaatgaaggaacatcccttgaggtgacccagcaaacctgtggccagaaggaggattgtaccttgaaaagacactgaaagcattttggggtgtgaagtaagggtgggcagaggaggtagaaaataattcaattgtcgcatcattcatggttctttaatactgatgctcagtgcattggccttagaatatcccagcctctcttctggtttggtgagtgctgtgtaaataagcatggtagaattgtttggagacatatatagtgatccttggtcactggtgtttcaaacattctggaaagtcacatcgatcaagaatattttttatttttaagaaagcataaccagcaataaaaatactatttttgagtctaaa

SEQ ID NO: 5 - DNA, 3042 bp, Homo sapiens
  source 1..3042: mol_type = genomic DNA
cgcccgccttcaccggaagactcggaaggaacctggagttctccgcaggcccgggccccgccctgagctttccagcggccgggaggagcggatcctcggggccaggaaggtgagcgcacctttcgctgagcacagggcggcaccgcgcgggcggaccccggattctccacccgcgacccaacgaattttcgccctatccggtaccggagacgaaagtctccttcttccgaaataccggcttcctctcttcgccctgccaaccacttttttagtttcttctcatctctcggaagcgcacgtctcctaagttaaggagtgctgagtaacgcgtgagggagttggggtgtctgcgagcacctgtgattgaagccccctcttctgtgatcagtcttcgttttctgtcttccggcagcctcagtttcccccccatgaagtgatggtgtgtgtgtgtgtgtgtgtgtgtgtgtgtgtgtgtgtgtgtgtgtcgggccccgtgtggtgccctctgtgcgcagcgagagctataactcaaggtgtgcacggggagagtgaagcgaccacgcacctgcttccaatcgggctcgggcgcgaacactcaggctgattcctgaaggtcgttttctgaaggaaaagacagagcatgcactagccacgggtgacattcccacccgtacaaccgcgtggtgggcgcgtacatccaacattgacccatgcaggcgcccgcccactgcgcacaccggtcgcagggcacttcgttgttgaacgttgggagcagcgtttgaaggccggatctctcctggcagtgcggattcgggaccggcggaagcagtatggcctctgcgaccgttatccctacttttcggggccgaccccagggccctcacaactcctcatcaccgcatatgtgagcgccgcccccacagggttttctccacgacctcgttcttggctaggtcgcacctctcttagtacctcctctctggccagaacgaatctttgactccgagctgcgcagtctacgcagacggggcaggatccactgcagttttccacaggcaaatacctgctggctccaccttaggcgagatgtggcctctcggggagggacccgttgtggacacgtttgcgcagccggtgaggtgaccagataataaccagggcagctttccttagccgggaacccaggtaccggcctaggaatccgtgaatacattcgcaaagtcgcgcgcgcgcgcgcgcgcgtgtgtgtgtgtgtgtgtgtgtgtgtgtgtgtagacacatacttttgtccttgtaagagtatgtgtacatctaaatgtgtgcgttttagacattagtccatttcattagtccatccatagctggtccaggggtccgaggcctgaagagtttgaaacactcaggcctgggttatttgaccgagaaacctggcggcgacagtgcagcggctgcatctggggacggcgaccccacctacagtggcaccgaccttccctctggctttccggggctctgtccgggccaggatcccaccactcgccccgccccgcggtcccgcgatcaccctgaggtcctgctgcagccgctctgaagagtctgtagcgacccccagccaaactctccagctaggaatgcccgaggctcaccgaaagctggcgctggggaggcctgggaggccctggagcggcgccgtgaggcctccgctgggcccctcccccacctaggccggccccctcccccttcccaggaaccccctcccctggcggagccccgggggccgagtgtgcgtgttcctttaagaggccccggggggcgcctcgcgggccgcccggggctggagggggagggcgcgggcgggggcggctggcgccaggcggccgaggctccacaacaaagctccggcccctgtcacttcgcatcggccaggtcccgcagacaggcgggggacgcgcgctcggccgcccctccctctcgcaggcggtctccggccagggcgtcgggcgggcttgggctggtggcgcgcggtctgtgcgccccgcgcttcccgcaacagtgaaatggggcgggagcggggacggcctgggccgggtggggccgcggtcctgagcctggcgtggctgcccttccgtcctccggccccgtcacctctcgcagggttaaggggcactgctgggaccttccccgggttgagcctccaggtggcagggggtccccgccgcttcctcctctgtgtgcagggccggggttgcgtgaccccgcgggcagtgggcagcaggaagctcgggctgtgcggccgcgtggcagagcggacgacggacttgcgtccgagtgacggggcgcgggctgcagactggcttaagccctcggtggcagacgaatgtgcccaggctaagctcaggggacgtgtgtggccccgtgctatgggcccgctgtgagggtgccgccaggccgtcgatcactgcctggacgtgaggagtgtggtggtgaaggacactccctggacagagtcgcttcccatcacggcttccccgccggaccgcacctcccggagccctggcgccagccagcccggtttagcggccggaccgggctcccccgcggtcccaggtctggttggggtgggggccgcggcctcggtgaccccagcccgcagcggcccggcccgtcccgtccacttaaacaaattgccgctgacaggcgcgcagtctctctggagccgccgccctcccgtcgcctccctcccgtcccaattatcccgcgcagggtggggccaactggctgggatggggcgggggacgcggggagagcgggcggctcgactccctcctggtcgcggggtggcccggggaagcgtctccgcagccacggcctgtgtggccccgtccctggtcttcccgggggatgcgagggcaaggcccagcctggcagctgtgggccctggaagggcgtcgttctgcacctaagggcgagatcacgcggccgagaaccaaggccgcatcccggatggacttcgggtgactttcccggagttctggggaatcc

SEQ ID NO: 6 - DNA, 3037 bp, Homo sapiens
  source 1..3037: mol_type = genomic DNA
cgcatcagcccaatcaggggagataaaactgtgggcactgaaacgttcccagttttcttttccaaagagtaaaaatcaagaccttaaaaatgcttaacaaaagttaaccacatgttctcacccacgtatggaagcttaaaaaaaaagtgatctcatagaagtaaaaagaagaacagaggatactagaggctgggaagggtggggggaaactggggatagggagaggttggttgaaggatacaaaattatagctaggtaggaggaacaagttctaatgttctacgccactgtaggatgaccatagctactaataatatacagtttcacatagctaggaggaggatgttaaatgttcccggccgggcgcggtggctcacgcctgtaatcccagcactttgggaggccgaggcgggtggatcatgaggtcaggagatcgagaccatcctggctaacaaggtgaaaccccgtctctactaaaaatacaaaaaattagccgggcgcagtggcgggcgcctgtagtcccagctactcgggaggctgaggcaggagaatggtgtgaacccgggaagcggagcttgcagtgagccgagattgcgccactgcagtccgcagtccggcctgggcgacagagcgagactccgtctcaaaaaaaaaaaaaaaaaatgttcccaacacacaaaaaagtgatatttgcgatgatgggcatgctaattaccctgatctgatcattttacattctatgtactgcaccatcactgtgtaccccataaatatgtacgattactatgtgtcaattacaaaaataaaaaaataatttaacaaatgtaacagagtagcggatatgaacaacattctaccagctgtgtcaagaaatcagtgtatacctttcaaagtaaccatagatttctaaagcatggagaaacaattcacggaagcctgctgattttgttgtattttgtcacaataaatagtaatagaatgattttacgtttaaaaaattacttccaaatatgaccaacctgcagttattttcagtttcggaacctgaaggctcactgtcccggggtttccttcagagctatttccacgttactgctaaccgcctgtcactgtccctcagacgatgccacaacgcagtggttttcgagttttaccaaagcgacagaatctttttctttttttaaaagatggaatcttgtgaggagccccaatacaaaaaaactagtgttttattatcaattaattttataaatttacatttatgacaatatttacaagctgctcaaagagaacaccgtgactgcgcagagcaggagttggcacgctatctctgcaaaagtccaagtcatcaatattttagactttgagggtgaaatggtctctcctcatcttggccttgtggcctgagtgtggatgtatgggagtgggtgtggctatgggctaataatactttattgcaaaacaggcagctgacccttgactgtttgggagagacaaaaagtagaaatcaaagctcaagatgacagtcctagcttcttgtagccctcagtgttctagttatcactccactttattttagttaaattgtatcaggaaagtcacgactgatgctggtaagaagttattgtaagtaccgaacacctgctttgcaagctcaggatagacttttttttttttttttttttttttttttttgagatggagtcttgctctgtcacccaggctggagtgcagtggtgtgatctcagctcactgcaacctccacctgctgggttcaagcgattctcctgcctcagcctccctagtagctgggattacaggaatgtaccaccatgcttggctaatttttgtatttttagtacagatggggtttcaccatgttggtcaggctggtctcgaacgcctgacctcgtgatccgcctgcctcggcctcccaaaatgctgggattacaggcatgagccaccgtgcccggactcaggagagttttaaaatgaatctagcagctagaaaaagtattaatggtgtttccctcaccctggcccaaattcatatgttggaaactaaaccccaatgtgatagtattaagagatagggcctttaggggtgattaagtcatgagaacgggaggctgaagagaggtgccttgccccttccctcatgtgaggacacagaaggctccatctatgagcaacacacgcttgccagacacagaatctgctggtgccttaatcctggacctctcagcctccagaactgtgagcaataaatttctgttgtttataaatcatccagggtaaggtattttgttgtagcagcaggaacagactgtgagaagcagaaaatttttatttcaaagtcacatcactatcgatatctaataattactgcctccttcatacctatttgaaaaaagtccaaatttctatttgcttgtgactgtgttttacatgatgaagttgttcccactgaattcggtggtacctttgggatggtctgatctgaatgataactcactctggaagacttgggagcttcttgaagagctaaaagctgtcctgctgagcaggtgtgtggaatgcaggagggccgtgtggaatggacagaaggtctctggtcatctcacatggaagtcccaaatacatttgcaggcactgattttttttaaatactcaaagttaatgtttgttttcctggcctctagctatacaaaattaattttgaataacataatccaaggaaatagaaacagatacatgacattaatattatatatattcacattttgctgtattttaaaaatcagatcttttctttataataaaacaacctaacacaaatgccaccccccatagtttaagttctgatctatagtatttccatctttctgatgcgtttgggtttagtatctttttctaatttctcaggatagacatagaggtcattattattaattttctcataagtgtacttaagacttcaaaattcatctagatattatcatttgagatacatttgtgatttgattctaaatatttt

SEQ ID NO: 7 - DNA, 2988 bp, Homo sapiens
  source 1..2988: mol_type = genomic DNA
cgcccaggggcagccatgcagaatcaaaggggcatccttcactgtcattattctcttttccctggacgggcccaaaacaagtttctgcttgggggaaaaaggaagttttgaaagcaaatagaactctcttgggaataaggagtgaaaacattaaaagaatgccccattctgacactgatgtctaggcatgcatgcatctgtgtttgggaatttttctgttcctacaagggagggccaggtttaggagcatgatttgacttattctgtaaatctaaggcacatcaaggatgctttataaaatgggactttttaaaagttacacttgttaacacttaatgcttttttggtcaaccaatatgaaaatatgttgtcacgtacttcgtagcttaaaggctagaattagaagttagtaaaattgaaatataatcattgaattgattcattaagtctttaagttctcttgcattaaggaactgctaagcattaattttccttggattttgctaatgtaattggacttaagctcatactcaaactgaggttatatatatgtacatgtatgtagaagaaatgatggcggttactgtagctgtacttgtgaaaaactaggatacttttcttggcagcattactaatgtcatatcaagagattgcctcaaaccagaagcccctgtcttgctcatgttagaatttaaagtagggttaatgtcttaaggttcccccagaaggagatttgagtgcaagttgtttatttaggaggtgatctcacatgaataagggagtgtggaggccagggaggggctaagacagttaagggaaggattcactcctgtccatcactgcttgagtgctgctgggttgtgcaatggagttctaattccctggcatttctcacctgcccatgaaggcctcagcaaatagaaaaccggcaggccaatagatacaggtgcaggtagttgcaagtcaggttaaagcgatggtaccgaggggaggggatggggcagagacagtgtctcttaccccggatgaaggaaggcttccctgcttttatgtgtttgggacctgggacgctttcagatgcccttgaggatttttattgagtatgtatctatctgtctgttcccttatgtctgtagattgtccccagctacggaaaacaagctccggctgcattaccgtagggccctcaggaacaatacagatccctacaagcgggccgtgtactgtatcattggcagatgtgacgtcaccgacaaccagagtgaagtggcggacaaaactgaggattacctgtggctgaaggtaggcactgtttcccctgcccacatagggctttaccccttttctgtgctcaagtccccgcaaagattttacctgcttaatgtatgatgccaatacagtgatcaggaccagtgggttcctcgtctcctgtccccattttttgttgtgtaattcccagctcataaccatagccttaaacacagcttctagctgacatcattgagcatggctgctgaacagctacaactctgtgcatgtggctcagggtgtcatttgtaccaatgcatgtgtttctcttggggatttagttgaaccaagtgtgttttgacgacgatggcaccagctccccacaagacaggctcactctctcacagttccagaagcagttgttggaagactatggtaagattctggacataaccacctttcccttctcttgtccacttaaggtgactacttcagttttcctctgggaaaatttttcatctctgaacttttgtctttcttccaaaactcctatagattgtcaaggcaaaacacaacaaaactaccattccaaattcaaataaagggcatgtggccttaagaaatacataaaacttatatggtcatacacaataatctgttttctctaattctttgaactgttctagtagacatatgctcagggagagaaaaagaagacttagctgttgcttcctagtcgatcgtaccagtcactagatctgagcacaaaggagagagaaacagcctttcttcttttttcccgtattttttaaaaactgagaagaaaagaagattccaaatagtggttaccagttgttgcattcagatttctgtgactgtgagtaaactgaaactcctttgaaatcttcatttctctccttgagtgacttaacagggtaaaggagataaacactctctgtggtccattttaaggtccttagctctgtttctctcccacctaatgcaagcagttggagttttacagcacagtcacagtttccagtaatgttatgaggtctagagaaggtggaggagccaggtcacatttcacatggcagtttactgtattcagggcccccttgatcaattcagactcaatctggtgctttcttcctgtccagcaagtcctgtgggctcacagggctgctgcctgggggttgggccaccagtgagccccttctttctaagttggttttatctcctctcctctcctctctcccaggcgagtcccactttacggtgaaccagcaacccttcctctacttccaagtcctgttcctgacagcgcagtttgaagcagcagttgcctttcttttccgcatggagcggctgcgctgccatgctgtccatgtagcactggtgctgtttgagctgaagctgcttttaaagtcctctggacagagtgctcagctccgtgagtatttgggattggattgacagtaatgtaaccacagcacgtcccccttggggcgacggtggccacaaaaccacaaccaataaggatttgagcaaagggtaccagtcattttagagcatgtggacagttgagctttttagatgattagtgttaagggttcctgcttcccccccaccccccagcattagtattcccttgaaagttaagtatataaagtgatgttcaaagtactagctttgtggccagtctgattgcctggaaaatgctgaagaagcagcccctag

SEQ ID NO: 8 - DNA, 3052 bp, Homo sapiens
  source 1..3052: mol_type = genomic DNA
cgggttgtcttaaaggcaatactgcctgcaaaaagagacatggtgtattctccagtactatatagatcaagcttttggcatatgacaatatggtattatctcccatagcactgctcctggatggccctcacaggtattaacctagtagggattaacctagaagtctgtctaacagagcttcccttgtagagctctagaccagtggttctcaaactttcatctgtgtcagaatcaccttgagagctaataaagatcactggagccagcctccttgaagtaggctagaaccagagcttttgtgtctctaacagtttctgtaggtaaatctaatacctagagtaggtaaactcctctagacgagtggttctcaatcctcattatacattagaatcactggggaaagaaggagtttttaaagcataaattgctgtgccctcccccagaatttctgattcagtaggtctggagtggaggcataagaatgtacatttcccaggtgatgctgatggtgctggttgagaaaccacaatttgaaaactattcttctgtaccaatcattcaggccttcaacgttgacactggcttgcaagagttctcacagattgaatcatacttcctgggatgattttttttcctaggaatttttataacactactttagaaataccagaatattagaagacattttactttaaagatgacttaattgaatattttattaagatttgttacttaccaactttatatacaacagtgattctaggctagagggaggggaggggaaactacaggagagaaatgccgcagattgttttgatattccacttacttcatccacccactctctcttttcccatcatacattaagtctactttgacagcttgcgatgtagagctttccttcactattctaattcattgttattgtgcttttgtgtttatgcatcatttagagttttgtgattcactgtagtttttaaccaaaaaaatttttttaatttgggatatagtactcattgttagtaattgaatataatatatattagaagtaaggagaagttcaaaaagtacgataatctgcttgaaatagaaaaaagattttattttgattaaaacaacacttttatgattgcatacatagataactttacaaggcaaaatattgcacagcgagaagaaatcagcattcttggtggaaccctcaatgatctggctaaagaaaaggaatgcctgcaagcatgtttggataaaaaatctgagaatattgcatcccttggagagagtttggcaatgaaagtatgttctgagaactgtggtttataagaaacgtttaaatgaaatgttaaatgttaaactatggtttaaaagaactagaatctgaataaaatatttgaattttctcaaatgtttttctagaagctggaacttcaaaatctgactttgaaatattttaagatagtcttaggaagcatgtgtacaaatctagtagctaatattttaagttgatttttctatcatgaattagtaattaatatcaattggcaagaactaattcagatatcaaaatataaagcatgacaataaagtagtgagactgatttcttcttaaaagcatattttcaggtagttaccctttgtaattgtgtttagaactaggaacactttttttttttttttttttttcaaacgggagtcttcctcccttgcccaggctggagtgcagtagcgcgatctcggcttactgcaagctccgcctcccgggttcaagcaattctcctgcctcagcctcccgagtagctgggactacaggtgcctgccaccacgcctggctaattttttgtatttttagtagaggcagggtttcaccatgttagtcaggatggtctcaatctcctgacctcgtgatccgcccacctcagcctcccaaagtgctgggattacaggcataagccgctgcaccctgccctaggagcacatttttacatcatcctcaggctttgagaatagatcatatagggctggtgaataaagctggatgataacctccatcccacatttttgttgttgaaaaaagatgttgccggccgcgtgcaggccgggtgcggtggctcacgcctgtaatcccagcactttgggaggccgaggagggcggatcatgaggtcaggagttcgagaccaacctggccaacatagtgaaacccccgtctctattaaaaatacaaaaaattagctgggcgtggtggcgggcacctgtaatcacagctcctcaggaggctgagtcaggagactcgcttgaaccccggaggcggagcttgcagtgagccgagattgggccattgcactccagcctgggcgacagtgcgagactctgtctcaaaaataaataaataaaataaataaaaggtgttgccaacaaggcagagatactgatattattttctagcttataaactgatttctgaaagcagttcctaagctgttttcacaaatatcttaagcaaaagcagcatcattggaataagggctttattagtttactttattactaaggtaactcattcattaatttatgtttccatccatccattcattatttcaacaaacatttgttgacatgtaccagatgttatgttagaaactgagggtgaggcaggggcatggtggcacatgcctgtagtcccagctacttgggaggctgaggcaggagtatcacctgagcctgggaggtggaggttgcagtgagcctagtttgtgccatcctactccagcctgcatgacagagcaagactctgtctcaaaaaaaaaaaaaaaaaaaaaaaaaaaaaaaggtgaatggtccgccttctcaaagcctctagtgtaataaggagagagataaagatactgttatgacagaatacattaagtgccataatgacatatgcacaatgtgttgttggaattgggcaaaaacacacctgattcagcctgggaattgggttaagggaggaggaaggtctggaaaaatcttccattaagtgatggtgcctggactaccctgaaaaatgactag

SEQ ID NO: 9 - DNA, 3057 bp, Homo sapiens
  source 1..3057: mol_type = genomic DNA
cgagtggcccagttccagtaaagcaacttaaccgagaagcaaaagcttgactccttaacccgggcctcatctattcagtgagctcttaatgtatttcaggcctgtggaagtaattctatctcttgagtccagagtccagtggctacttagagactaaggtagttatacctagaattttgtttaaaatcacatattggactgtagaccctaatattttttctattcatgaagattagtcccatggtaacctttccatttacttttagaaaaagtaaaaactggccgggcgcggtggctcacgcctgtaatctcagcactttgggaggccgaggcgggcagatcacctgaggtcaggagttcaagaccagcctgaccaacatggtgaaaccccgtctctactaaaatataaaaattagccgggtgtggtggcaggtgcctgtagtcccagctacccgggaggctgaggcaggagaatcgcttgaacccgggaggcggaggttgcagtgagacgagattgcaccacctcactccagcctgggccacaaagcgagactccgtctcaaaaaacaaaaacaaaaacaaagtaagaacctcagaaatgagactcttacccatgagaggtttagtcatctaaccgatcatgtctgtcctgcgccctttgtgcttacaacctgccgatccttgtctgtggtcttaaggcaactgtgtgttgatctcggagtgttttcgtgatgccccagtgtgctccctgcgtgctgtggtggaggtggcgctcccagcctctcccagcgagaccctctcctccccagcttccctctcgccccacaactcccacgcttgtctgacaggcctacctgggactcctggagctgtcagccgcccgggagaagcacgaggagttctgtgtccccatggtcatggttcccgctactgtgtccaacaatgtgccgggttccgatttcagcatcggggcagacaccgccctgaacactatcaccgacgtaagtccgtgtgcgccctgccaggcgggcgccggctgacgctaaccccggggccccggccctttttatctaccagtgcgctagaaatagccttttacaaataccctgaatgagagcttctcgttctttttttcccccagaaaagtatgttttaagactctgaaaatttttgatctcactcccagagagttttaccacctcttcttctgtgtggccaccagggggacgtagtgtggccgagactccaggggtgcccgtgagcacccgaggcgctgaggagggctgggtcgcagtctcctgtgattgtaccagcattaaaaatcgctgtgtgtgtgtgtgtgtgtgtgtgtgtgtgctgagcctaaattttctttgagcctccaatacccattatgatgaacccctgccttgatgctgagggtagaaattgaactgaatattttataattttattcattgccctgaatgcaccattgcatttgttatctctctggtcttggctgttgacctcattttcccctttgtaaactggggatgttaaattacctctaaggcaataattggtgctactttagtttttttgccaagagacaataataaaacatagaaatatattcttctttttttctttgtgggacggggtcttactctgtcacccaggcttgagtgcggtggtgtgatctcagctcactgcagcctcgacctcccgggctcaggtgatcctctcacctcagcctcccgagtacctgggaccacaggcatgtgccaccattcccggctaaaagaaatatacacctattcccatgtttgtgtgtcacgcttggtaattgatgtgggagtttgaagatccgtacctaacacagaaagcatttcatttttttaaaatttgatgtctaaaagtttgtagtaattctcaagttttaatttttcttgtgagacttggttctcatgaatatttttcaaagatattttttcttgtaaaaccttggcatgaaacttatttctagcactggtaaataaaaaaacaagcttttaacatacagctcatatggtaagtaatgcttagcactcgtttcttgcttttctgagcgttttaaactttcttcactttctttgcgaaggaaacctgcccaggttttcctgtgttcactggctttgggggcaactttcaccttatttttggcagttgctaatctctgacctagacgttgcttctgttctcctggtggtgggtgtcacggctttgctgctgcggggctggcccggctctggacctaccttcgcactgtgaatgtgaagatgagcctctttcacagactggattccgtcattgctttcactgctctttcgcctgctttagctagatttttgggtctgtgaaagttgggtgtgcaatgggagggactgaagcttcttttttccctaattgttacctaattggaactcgcccagagggaacgggtggagaatttgagagcggtcgctgcagttagctgagtttctttttaattccagggtcctctgctataaataactgttttttttttttttttttcagattgtaaatatgtaacaaatgcatagggtcaaatttatgaaaaccaaaatacgtggggcaaaaacaccccacaaatgatcatttccacctgcttttacttcccttggagggattgtgtgatttattatgcgattgttttaaatgcagtttttcattcattcgagtttctcgaagctaggttaaacaatttctttttttttctttttttttttttttttttttttttttctttttttggagacagggcctcactctgtttcccaggctggaatgcagtgctgcaatcgctattcactgcagcctcgacctcccaggcttaggtgatcctcccacctcagcctcctgagtagctgggactacaggtgggtgccaccgtgcccagctaattttttgtatttccatagagacggggtctccctgtgttgcccaggctggtctcaaaacgtctgggctcaagcaatccccctgtcttgggctctcaaagcacaggggttacag

SEQ ID NO: 10 - DNA, 3007 bp, Homo sapiens
  source 1..3007: mol_type = genomic DNA
cgcaacatgatgctctcaggcaggaaccacaacagaggacccacagcagggatgtgacctgtgaggcccaatgggtgtcacttgtaattgtgaactgtcactgttttgattggccattgtcttgccctgaaaagtggtaattattccatacggtgacacacggagccctgcacctttagatgcgctgaaactcccttggagcacagggccaaggccagaggggtcagcatgggatgttagggtctggccagcacgactgagatcaaagggggctctggtttgttggatcctcaagtgtttgcagttgtggggccccaaaagaggtggctgtggtgtggagaaggggccctgaagggacttctgtgagaacagcccccttatggtcgggggaggaccagaccttcctggtctgcagggagggctatgcactcccctgaagttccccgggaaggtggacatggggagtgaggaccctgtggactgtctcgtgctctgaggatgtaaggagccaggacaggatgaaaggggcacgtacctcccctgcttgtctgacgctctctacagaggacatttaccagaaacttgaaaatgctgctgtaaaaaagctgccacggagctgttgtgtttggggcaactagatctgaccatggaggaggctgtaactgatcgctttcaatgaacttgacgcctttaaattctaagggaggtggagattttccactgagacaaggcgtcctgatgcccccatgaccgagggtcacaccagcagtgtctgccatggcacacgtgccccagactgtgtcgcctgcttagcagaatgcagtggggctgctgagagagacacttgcagccctgcatctgggcctttgttctgcttggggtgcggcagagaggaggaacacactcatgattggggtggtgtgctgtgttggtgccgacctgaccatacggtgtccatgagctgaggctgtgtgccgctgacatgactgccttcatctcagaaggaaaaatacaagggaacagtcacatttgtttacaggtccaaatggtgacaaagtggtagctatgttaggaaataagcggaaatgataatttttttttttgagatggagttttgctcttcttgcccaggctggagtgcaatggcacgatctcagctcactgcagcctccgctgtctggaagcgattctgctgcctcagtctccctactagctgggattacaggtggatgccacaacgcccagctaatttttgtatttttaatagagacagggtttcaccatgttggtcaggctggttttgaactcctgacctcaggtgatccacccaccttggccttccaaagtgctgggattacaggtgtgagccagcgcacccagtggaaatgataaattatgttttctggcaacttcctggaggttaacagttcaacaccatgttttttcaaaacaaacctttactaaaattttagaggcaaagacatatccattgcgggaagtcagggaccctgaatggagggactggctggagccacagcagaggaacataaattgtgaagatttcatggacatttatcagttcccaaataatacttttataatttcttatgcctgtctttaatctcttaatcctgttatcttcgtaagctgaggatatacgtcacctcaggaccactgtgataattttgttaactgtacaaattgtaaaacatgtgtttgaacaatatgaaatcagtgcaccttgaaaaagaacagaataacagtgatttttagggaacaagggaagacaaccataaggtctgtctgcagggtcaggcaaaaagagccatatttttcttcttgcagagagcctataaatggacatggaagtaggagagagatcactaaattcttttcttagcaaggaatattaatattaataccctgggaaaggaatgcattcctaggggaggtctataaatggccactctgggaatgtctgtcttatgtgattgagataaggactgagatacgccctggtctcctgcagaaccttcaggcttactagggtggggagaaactctgccctggtaaatttgtggtcagaccggttctctgctctcgaaccctgttttctgttgttgaagatgtttatcaagacaatatgtgcactgctgaacatagacccttatcagtggttctgcttttgccctttgccttgtgtttgttggatgcttatcagtggttccgctttttccttttgtcctgttccctcagaagcatgtgatctttgttagaccgttattagtacgtctgctttttgccttttgaagcatgtgatctttgtacccactccctgttttacaccccctcccgttttgacacccttaataaaaaacctgctggtttgaggctcaggtgggcatcacggacctaccgataggtgatgtcatccctggtggcccagctgtaaaattcctctctttgtactctttctcttgctcagctggctgacatttatggaaaatagaacctacgttgaaatattgggggcaggttcccccattacatatcttcaaaaggtttaatttgaggttggctaggattatattttacattattgttaggtgggtaaacaaggctcccctctgctcaagtccttgaaggcccaggaccccccagtttcatcctcttactatgggcatgacattcagttgtgacgtgaagagcagtgtggacccggtggaaacacccaaccatgaaagttaaaagctggagccttttagacacatggagagcacatcacagaggcaacgcccctcacaggttggagggtttggagtgcaggggagggatttgcagtagttgggacttggccaggaggaggggctgttaggatggcccctaagtgttttgagggaggagaggcccactcaagactgtggggcccatggacaaaatacaaaggccaggtcctcactccctgcttagtctctctggcaccagagccaggggctgttgggcaccc

SEQ ID NO: 11 - DNA, 3041 bp, Homo sapiens
  source 1..3041: mol_type = genomic DNA
cgatgagtttattaacatgtgctttttatttagggtatgagctacagttccgattaggcccaactttacagggaaaagcagttaccgtgtatacaaattacccatttcctggagaaacatttaatagagaaaaattccgttctctggattgggaaaatccaacagaaagagaagatgattctgataaatactgtaaacttaatctgcaacaatctggttcatttcagtattatttccttcaagggtaagtcaggtgttttgtttgtgagaaaaaaagttaatttgttctgtaatttgaagtcacctaacttgtaaatgttactgtatgaaccatggcagtgcaatttttatagtgcttccttgagatgcaaatagaatattctttgatttctaggaggtaattttatggtccattgcagagctaaagtatcaagtaaatgtattttaagtaacatcttaaaatgtagtaatttcatgcaacctgattataggttgctgtttatttgcgtgcccttgttattactgataggttttagtatacttatatttcattaaaccaacattcttggatattttgtgtattatacatgtaattatgtagattgtgaaagggtaaaagtagcttttccattaagttttgttgcaacttttaaaatgattttatgtgcttagaaataaatacattttatttgggacaattaaccttttagttagagtcagactatattatatgaggattttttttctatcactgactgaaaagtttttgttttgttttttcccttagaaatgagaaaagtggtggaggttacatagttgtggaccccattttacgtgttggtgctgataatcatgtgctacccttggactgtgttactcttcagacatttttagctaagtgtttgggaccttttgatgaatgggaaagcagacttagggttgcaaaagaatcaggtaatgtcagcttgctttctttttcttatttaaaaaaataaatgtaattatcctctgtgatatagatttcaaaagttttgtgtattagtccattctctcattgcagtaaagaactacctgagactgggtaatttataaagaaaagaggtttgactcacagttccgcaggctatacaggaagcatggctggggaggcctcaagaaacttacagtcatggcagaaggcaaaggggaagcaggcatgtcttacatggccagagaaggaggaagagaacaaagtgggaggtgctacgtgcttttaaacaaccagatcttgtgaaaactcactcactatcatgagaacaagggggaaatccacctctgtgatcaaacacctctcaccaggcccctcctccaacatcggggattacaattcgaatgagatttgggcagggacacaaatccaaaccatatctttttgcctctatgtttaattttgtttcttattatttagtaatataagtagatagaaccatattaaaaaaaaattttttttttttgagacggagtatcaccctgtcacgtaggctgcaatggtgcgatctcagctcactacaacctccacctcccgggttcaaacgattttcctgcctcagcctcctgagtagctgggattataggcacctgccaccatgcctcactaatttttgtatttttagtagagacggggtttcaccatgttggccaggctggtctcaaacttctgacctcgtgatctgcccaccttggcctcccaaagtgctgggattataggcatgagctgctgtgcttggcccatattacatttttgatacttaaccatttttaacctataaaaatggcaaattttgtggttcagcttaagaaatgaaggaactccataatgaaacacttatcatttctaagactttaccatataaaaatcagaaataagctattgaaaagtgaaggaaaatgtattatcattatgtatcattttaattcaacaaacattggttaaccatcttttgtgtagaagacatgtgctaccataaataccaagagcaaaatgaaacttgtgtttcattttggcgcaatctcggctcactgcaagctccgcctcctgggttcacaccattcttctgcctcagcctcccgagtagcttgggactgcaggcgcctgccaccacgcctggctaatattttgtatttttagtagagacagggtttcacggtgttaggatggtctcgatctcctgacctcatgatccacctgcctcagcctcccaaagtgctgggattacaggcatgagccactgcgcctggccttttttttttttttttttttaagacagtgtctctgtcacccagactggagtgcagtggcctgatctattttttgtagagacaaaagtctcactgtgttgcccaagctggtcttgaactcctgggctcaagtagtcctcttgccttggcctcccaaagtgctgggattacaggtgcaaaccactgcacctgatctcaatattaattttctgcttttaagttggataatacatgaagaaaggaatgagaagttcactgacataactaaaacagaatacaagtactatggaacattaaaagtagtagaaacacgtgttgatatactcgtagaagataaatttactacatgttaagtatataaattttctaataggcagtgtgtgtgaattttttcaaatattatctcattatctctgtcttgtatatgaggacacatatcttgaaagatttaaataaacttgcttaaagtctcttgtggtacagttaggatttgaacccaagtgtttgacctcttttccagtagcatgcttgccttgctatttataattacttaagaaagtttaaatttatattttcttcattttaggctggttttgtttgtttgtttttacagtggtctttcctttatttgctttgcaggctacaacatgattcattttaccccattgcagactcttggactatctaggtcatgctactcccttgccaatcagttagaattaaatcctgacttttcaagacctaatagaaagtatacctggaat

SEQ ID NO: 12 - DNA, 3068 bp, Homo sapiens
  source 1..3068: mol_type = genomic DNA
cgacacagatgctggacttgagagaacaaacccagaatatgaaaatgaggtggaagcttctatggatatggatcttttggaatcctcaaatataagtgaaggggaaatagaaaggcttattaacctcctagaagaagtttttcatttaatggaaactgcccctcatacaatgatccaacaacctgttaagtctttcccaacgatggcacgaattactggacctccagagagggatgatccataccctgttctctttaggtaagacatgtttgccttttgggaaataaatttcacaaatcattggagacaattttatgtggttgattttgctttttatctgattgtaggtaacttatttatgtgtaaggatacttgatatttcaaaacggttatttagtagtggaactgagaagtatgttactgtgggtgagcttatattgtgttagttcttaaagcaaaaatgggaacttcagtgaaagattttagtaattaacaatgatgcttgtataagcatgtctatgagcaagaataaatgagaaactgctgacttgcttctgggaaggtggtaacaaaggaatggtgtaggaaggagagctcttctgtgtgaacccatctgtacttactactcttaatacattgtaagttaaaattatattttactagcttaattttacagtgctggttaaagatgtctttaagtttccattactacttgtttctgccatctacctctctcatctgttgatacagttttgccattgttaggaccagcatccctagtagattttttattttgttttgagactttctttcttaccatttgcctgtaaataatttcctaacataaaaatggaaaaatggcatttgaattattttattacttatttttgtgattaatattttcattgatttggatggagcatagtgcattcccaggggatgggatatgtgtccagtctaaaacctccacttatccaagttcctgtttttagctgaaactgttacaccttgtcttagttttgagtttcctaaaaggataacttgagtcaaagtcttgggtgcaggttctttgaaagattatcctaggaagcagaaatgcctgaagagagtaagataaggagaaaaaccagtaaaggaagtgttattatacttattgctgtggacagctggggctcatcctactggggatcctccgaagaactggttaaagtgtatctcctgcttatcctcctaaaacattcaggctgggcattcgtctaccaactctcccctttggttcaaggatgcccacaagaaacttttaactcttttatgcttctgagctgttcctgcttgtggtccgagcaccctttaatccctttggggggaaccctgagaaagaaaggtagagaggcccaaagtgaacacttgaggccagatactggcaaccctcacagattgtgtactgggaaatcaatgggtcagtgatgggaggttggggagcagtaatatgtaagagatgggcagagaatgcatttaggcaggatacttagaaggaatagaaagacaaaatgagaagcaggagagaatagaaactaaggaagcaaatagttttaggaaccagtgaatggtttgttgtgatactgtgcagaggttcagaagataaggataggaaatcatgtattttgtaacatagattgcaaatggggctctggcaaaagtagtttaatgtagcagtgggagaggaagtgtagatgaaaaaccactggccagtaaggatttgaaatggtgtaggccactgttttaagaaatgtgggtggatcacctaaggtcaggagtttgagaccagcctggccaacatggcaaaaccccatctctactaaaaataaaaaactagagccgggtgtggtggctcacgcctgtaatcccagcactttgggaggctgaggtaggcagatcatctgagttcaggagttcgagaccagcctgaccaacatgacgaaaccctgtctctactaaaaatacaaaaattagtcgggtgtggtggtgggcgcctgtaatcccagctacttgggaggctgaggcaggagaatcatttgaacctggaggttagagcatgcggtgagccaagatctggccactgcactccagcctgggctacagagtgagactctgtctccaaacaaacaaacaaacaaacaccggccaggcatggtggctcacgcctataatcccagcactttgggacgccaaggcaggtggttcacctgaggtcgagagttcaagaccagcctgaccagcatggagaaaccccatctctactaaaaatacaaaattagtggggcatggtggcgcatgggtgtaatctcagctacttgggaggctgaggcaggagaattgcttgaacccgggaggcagaggttgcagtgagctgagatctcaccattgcactccagcctaagcaacaagagcgaaactccgtctcaaaaaaataaataaacaagtaacaaaaacacacacacacacagacacacacaaaaactagccgggctttggtggaatgtgcccgtaaacccagctacttgggaggctgaggcaggagaatcctttgaacccgggaggttggaggttctggtgagccgagatcgggccactgcactccagcctgggcaacagagtgagatgctatctcaaaaaaagaaaaactagccaggtgtggtggtgcatgcctgtaatcccagctaactcgggaggctgaggcaggagaatcgcttgaacccaggaggcagtggttgcagtgagccgagatcgtgccactgcactcctgcctgggcgacaagagcgaaactccgtctcaaaaaagaaatttggccagcctgggcaacatagggagaccgctacagaaaataaaaaatcaaaaaaaaaatagctgggaatggtagtgtgcgcctgtagtcccagctgctcaggaggctgaggtgggaggattgcttgagcctgagaggttaagggtgcagtgagctgtgattgtgccactgcactccagtctgggcagcagagtgagactgtgtctcaaaacaagaaatttg